European Patent Application EP 4 650 436 A1, published November 19, 2025. Title: NOVEL PSEUDOMONAS STRAIN. Applicant: Bioomix A/S. The sequence listing filed with the application follows.

SEQUENCE LISTING (17 sequences)

SEQ ID NO: 1 - DNA, 1532 bp, unidentified
  source 1..1532: mol_type = unassigned DNA
tgaagagtttgatcatggctcagattgaacgctggcggcaggcctaacacatgcaagtcgagcggatgagaagagcttgctcttcgattcagcggcggacgggtgagtaatacctaggaatctgcctggtagtgggggacaacgtttcgaaaggaacgctaataccgcatacgtcctacgggagaaagcaggggaccttcgggccttgcgctatcagatgagcctaggtcggattagctagttggtgaggtaatggctcaccaaggcgacgatccgtaactggtctgagaggatgatcagtcacactggaactgagacacggtccagactcctacgggaggcagcagtggggaatattggacaatgggcgaaagcctgatccagccatgccgcgtgtgtgaagaaggtcttcggattgtaaagcactttaagttgggaggaagggtacttacctaatacgtgagtattttgacgttaccgacagaataagcaccggctaactctgtgccagcagccgcggtaatacagagggtgcaagcgttaatcggaattactgggcgtaaagcgcgcgtaggtggtttgttaagttgaatgtgaaatccccgggctcaacctgggaactgcatccaaaactggcaagctagagtagggcagagggtggtggaatttcctgtgtagcggtgaaatgcgtagatataggaaggaacaccagtggcgaaggcgaccacctgggctcatactgacactgaggtgcgaaagcgtggggagcaaacaggattagataccctggtagtccacgccgtaaacgatgtcaactagccgttggaatccttgagattttagtggcgcagctaacgcattaagttgaccgcctggggagtacggccgcaaggttaaaactcaaatgaattgacgggggcccgcacaagcggtggagcatgtggtttaattcgaagcaacgcgaagaaccttaccaggccttgacatgcagagaactttccagagatggattggtgccttcgggaactctgacacaggtgctgcatggctgtcgtcagctcgtgtcgtgagatgttgggttaagtcccgtaacgagcgcaacccttgtccttagttaccagcacgttatggtgggcactctaaggagactgccggtgacaaaccggaggaaggtggggatgacgtcaagtcatcatggcccttacggcctgggctacacacgtgctacaatggtcggtacagagggttgccaagccgcgaggtggagctaatctcacaaaaccgatcgtagtccggatcgcagtctgcaactcgactgcgtgaagtcggaatcgctagtaatcgcgaatcagaatgtcgcggtgaatacgttcccgggccttgtacacaccgcccgtcacaccatgggagtgggttgcaccagaagtagctagtctaaccttcgggaggacggttaccacggtgtgattcatgactggggtgaagtcgtaacaaggtagccgtaggggaacctgcggctggatcacctcctt

SEQ ID NO: 2 - DNA, 14515 bp, unidentified
  source 1..14515: mol_type = unassigned DNA
caggatcctctgctttgtatcagggggcggacattttagttttgcaagcatgcgttgagaatagttcgaagtaaaaaacctaatggttatcggaaaaagataaaagagtcgcagttcgctgcgcacgcataagacgtatcttattgatttttatactattaagttagcgtcagctgagtagctcagtgatggggcgccgagatgagcagttccttcatttagtcttttttgccgttggtggtggaaaccaggcgcgagtagttctagcttatgccccggactaaggagcggttactcgtggctaatttaaacagcgcgtcgtcatcaatcgatattctccaccatcggcgtgcaatggaacgttgggatatctttcgaagatataagcaaggcgaattacctatggacgtcgccatgcgagtcatgaatcttaagaagtctatgttttacaggctgttgggggttgtgaatagatctgctaactacgagtgcttactgcccggcaataaggggtgtaactctggttcgaggtacttaggaaataaggttgagaaactcatagatgatgcttatgaggatcattatgaaggatcgtctgcttcttttgctaatgtttggcgtcaactccaggcgataacaaaagtttctgacttgaaatgcccgagctaccatgcagtccgtatcagaattttagaaaaacctgaaatcgagaggttcaggaagaaatacggtgttgaagcagccgaccaaaagtactcgccccgtcctggcagtaagcaaaccaacaggccgttagagtgggtgcagattgatcacactttagcagacgtgatgttagtcgattcgcaggatcgaacccagcttatagggcgcccttgggtaacgctagcaatctgtaaacacacccggctgattctcggattttatctttctctcctgcatcccagtgctgtgagtgttgctatggtcattgggaattctgtggcgtcgaaatcatcgctgctaactaagttgggaattagtgaaaatgcactcccgcgccatggcttgatggagacaattcatacagacaatgcggctgaattcacctcagatatactcaggagcgcttgcgaatcacatgacataaaactagtgtctcggcgtcgcaagcattacggcggtcatatcgagagacttattggcaccatgatgaccactaaggttcactttctgagagggactacattctccaacgttctcaggcgccgtgactattctccagaaaaaaaagccgtactcacattccaggagttctgtaaggacttcgtagttaatgtgagtgtttataattctacaactcatagcgcgcttcaaaataaatcgccgaatcaagtgtgggacgaatattacactaaaaatccacgcccgaaaataatagactcatcggagctagaaagctttcgaatagatttcttcccgcaacgccttaaaaaaatacaaccctacggaattgaaattttggggcggcgctattatggcacgcccctgaaaggtttagtggggcgtgaagtcttggtgaagtttgacccatatgatcttacgcatgtatttgcgctgttgcaggggagctatcagctcataccgctatcttataattataagtcgcgcagtttggactatgagatgtatagatacgagagaaatcaaaaaggtgttaggaacggaacaattacggaggacgaggcgctaggcctcatgatcgaagctaaagcggacctggaagctgcgcaacaaaaaactcaggaagcgaaaaaggggaggaaatccgaggcgtctagaacccataaagctgcgaaggaaattataccggccaattcaattcctggttccattaatccgccactagctgtccagcatgatcggataggtattctcgactatctcatagcttcgcggcctgcagacacccatgcggaagatatcgactttagtagtcaaccaaaaatttatgatggagacttaaagtgagcaacggatttgaacatgtacggcccgaacgtcgacacttattcgatctttccattgagcttcgcagtctcgcatgccgtgccgatctttggattaatgcccctcacgccgaaagagttgttaacaaaatcggtatgatgttaaaggtaaaaaataaggttcaagcgccatgcttattggtatatggacgaggcggttctggaaaaaccacgatttttcaacgcttgcaatctctttatgaaaatgccgatgaaaagcttgtgtttgttaatatgcggcagaatccaaataactgggcattccgagagctgttattttccgcgtttgacatagcggtgacaaagcgcgcacgtgccactctagatatttcagcacaattgcgcatgctgatcgagacccggaatataaagggtatcgtgattgatgaggtgcatgatgcattgaccctgactgctgtgcagcaaaagataaatttatcgctgttgaagaatttgtccggcgccgattataacttgtctgttttcgcatttggcacagagggggcggaggaagttctcagagctgatccacaactggccaggcgttatgcaatgcaccctctgctagattggcaatggggggatgcattccgtaattttgtagcgagctatattaacttccttccgctgcgcctagccactgacctgggaaataagcagctcttggtggcaatgttcagcaactcgaaagggattatggataatgttgtaaagctcttgcaggtttgcgcaagcgctgctgtgcttgatggaacagagcgtataacgctggagcacgccaataatgtcgggctgttgtgccatgacttgggcgtagcgtgggagtaagtttgttgtcagacgctacagaaaaaatcgcatcagccctgtcctttcagccggtctggcaagatctagcgccatcccttgatttgatggctcgtattgaagagttttctgaatgcgatgccgggccgagagttttcgtcgcatatggagagccaggctgcggcatgacgagggccttgagcaggcacttctcaagcgcagcacctcattcagtatggcttggtgccaagctcttgggtacgaaagcaaccttgtatgaccggcttgcaagatatatgggcgtatataacgtgtgccacagattggatcgcttgccgaagtatttgctgagaatgttagagctccggcgagtgcggataatatatgtagatgatgctgatcagtttatgttggatcgcatggctgctgaaagttttattgcagatattgcactgctcgcaaggagttctcctgctttacattttgttctcagcataaagtcatctcgggcggacgtagaacggtcaagcttgcttaaaagcctgcactgtgtaacccataatttacagggcttaaatggcgtcaacagcaaggagttagctctcgcaatgttaaaagaactaaacgagctaaacggtacgacgattaccttagccagtgaggtttctcggtgcccccccccggggagaggcctgggcgaattagtcgattgggtaaaattggcatttgcaacggcatggattacagaaaaacaaatcgatccgcatgcctcatactctaaactatggaaggtgctggatgattttcttgagtgaaccaccattacccgaagaaacgatggtctcatgggcatggagagtgtttaatgaagtcgactgccctaccgagtggatagccttacatcaggctttctatgcttcgcatggatgtgatcctgactttaattttctatcaccattcgctcttgagttgcagagaatcactcaattaaccgccagtgatttgcgtgagagtttctcggtaggaggggcgttggtgattccgaggaaagccaggtctgcttactgctacgaatgcctagaggatagcgtaaggcaagtagggcttccttcttggaagaggtcttggtgctcgccattcatccccatttgtcaaaaacaccagcatgttctgtctgataccctcaatagtgatgccaaatattatgaatttcctgcattggcgttcatcgaaggcgcagagtcgtcatattcggcgagaggagggcgtctatctaattattccaaacgctggcatggggaaagatatatggaccccgcggttcaatctcagcactggtactgtagttttctgagttctggttcggagtcatggaggttttccttaaggcgattatgggaagtcatttttattgctctgatggcgtgccatgttgctcgcttaggaacttggaaaggctgggcggcaggcgaaactggacccggcagatcaaccgccagagagaaacgcaacgcaacaggttccctgttgaaagagggcttgtacggttcgatctccacacgaatggaagcgttgttctactgcggaatggtattcggcgtattcagattcatgtcttcggaagatgacgttttcggctatgcaccaatggatccactggttttaggacgccgaatgcgccgagacaaaccagaaatttcgctatggttggttggatatatggaacgtcgtcatgcattgctccttcccgctactaagcaatttctagagggactcaagctctcacctggctcttatgaccatcgattcaaatggtgagacaacttgctgaatagattgatcacctatttcatttctaatgtcggccaaaataaggttcggctaggccgagcaggcataggagcgcgacaaaccctacagcctaatcattctcgagtctgtttgcgaggctcttccctgagttgtggtgacgcgggatagtctcatcggagtcggtcagagaacaggtgcgtttgtgctgttctgggcgttgtcagcgtcgtcctctagcgaagattgagttgtgaatagctgggtggcacgactacctagcagcgatcctgcctgaaaatagcccatcaccgtactgacactgcgatgttcggtcatggccatgatttcaccgagtggcacaccctgacggctggcttcggtgacgaaacccgagcgcagactgtgcgcggcccaatcaccgtcaaggccagctagttgggcacggcgtttgacgatccgcgccacctgatcccctgacaatcccttggtggcgaccttgccacctctgtacaggcggcggaacagggggccggtctgagcaggggccgcctccagccaagtgctcaacgcgtgcgccggcgccccttgtattggcttcactcgacgcacaccactggtgtcggtcttggtcgcacccagggcatacaaccaggtgtcggcatctagctggcgcaggtcctggacctgcaagcccaccacttctgagcggcgccgaccgccgccactccaggccagcagcaacagcgctcgatcacgcaccccgcgcaccccgtcggtgcaggtggccagcattgcctgcaacggttctagcaccaccgcggtcttcttgcgtagtgtcacgccctggcgggtttgcgccttgcgcgcctcgcgcaagagggtcttcaccgctgaggcctcgcacgggttgtcccactcgttgaggcggtgccacttggccaacactgccaggcggtgactgaccgtgttgaacgccaatggcccaggcttacccttgaccccggcggcgactagcgcggcatcgagctcggccggcaataaatggctccagccaccagtgccatccgggcgggccaggtgatcgacgatgaactgcaccgcgacctccgggggcaaagcgccgtcaccgagtgcccgaccgtagcgcaattgcagccagccggcccaataggcgagggcgctgcggtagctacgcacggtattcgccgcagtgccggcagcgatgaacgcctcagcggcgaagcgcgtactgtccgctagccgaaacaggtcaagggggactggcgtaggtaatttcgtctcacttgtactattcataacattgcacgtattaagaattgagtgggcgaaaaacaggtccggataagattgcattatcagacctaatatagcggagggcaggccatggcggtaggtgtaccggaaaacgacgtgttcgccgcggcggacgcggtattggcccgcggcgagcggccgacggtcgagcgggtgcgtctggagctcggccgcggcagtccagcgcgggttggctccttgctcgatcaatggtgggaacaactagccgggcgcttgcgtggtgaaacccggctgcccggcctgccgacggaactggcacaggccttcgtcgccatctggcagcaggcgaccaccctggctcagggcgtggccgaatacgcgttggccggccagcgccaggttttggcggaggaacgcgagcaactggtggcactggaggcgagggcgcgtctggacgtcgcacaggcccggctacagaccgccgaggcgctgggggcgcggcagagcgccgaaactcggttggccgatctggaacagctgctgatccagcgctcggcgcagatcgacgacctgcgccagcagcgcgaggaattgctcgggcagtgcgacgaagcgcgcgggcaactggtcgaagtccgccagcaactgcaggacagtcgccagcaggccgagcaggcacgcgaagagcagcagcgctacacccgcgacgtcgaggaccgggcatatcgggagatcgatcgggcgcgcgaggagagcaaagccttggcgacccagctcgaggaggccaatggccgtttgcagaccttccagcagacgttgctagcagggcaggcagagctggccgaaacccgggaacagcggagcatcgcgcagacccaggcgcaggcactgctacacgagcgggaacaagtgcaccagctgcaggctgagcggtgccgccagcttaaggagctgcagcagcaactgcagcgcacccatggcgagttggccagtgcgcgtgagcaagcagccgctgcgcaggcccgcgccgaaacgctgcgtcagcagttggctgactccggcagcagcaatccagtgcccgggggtagtcagcggctgcgcaaaggtacgccgagaaacagctgaggccggtcaggtgaccggtgttcgctgctggccgccaactgcgggaacagcggcaacgcaccaggctgcataccgaaatttggccgatttatgccgctcacgattgatcggtataagtcggctgcttcccttggtgacaggccagagccggcctaagggactgtggttgttcaccagctggccccggcgttcgccttcaacaaacctgcatcaggccgtgcctccccattcaagggcttgaagcacacggcgaacttgtttggctccgatttcggtttcgcagagcataatcgacccattgcggacgttcggcactgggattcgagattatttttttgccccacgttgatggaatctcacgctgtgccctcaacccaaattcaggttgcaggagcaaggaaactacgaagcacgccaacaatttcttgaagcgccgtatcgtttctgcgcatcaaatatccaaagacctgtttctgcgtcgctagccccgtacaataaaatcaagcaacatatcaaatatagcctaattgtttaaaaattttctgatagatatcacgtaccactttacttttattttcatggtatttctgaatatctaagctgcaatctttaattgcctcaaatttggcgtccgcataaatcttgcagtccttctcagactgtctaagccaatcacggaaaagcaagtgccgggctgtttcaggggtatcccgagtaaaaacatgcagattaactctcggattatcataatggaaaagacgatggccatggaagcggggctcacgaacaattagtctatacccaagactttcaagcactaatacatatgttttttcatcagcagcatcagcaaccgtcagatcaatatcaataacaggtttagcggctaagccaggtactgccgtagaacccacatgatcaatttttagtagattcgaacctaatttattcttaatttcagattccaatgttgaatatatttccggccacgagggttcataagcaacaaccgctacattctcaatcggcggtacgccattaacaaaatagctatcctgaggatcgatgacatagtgatccattatttcttttggactaatcataaacggatacctataaaccataaagatgatgagcgatagcttacaagaggtgagtttggatgtctctcaaatgtccgcttctggccggatagcgccccccacgctgtgtgactgatccatccttgtcctccctcaacgtggaggacaaaccatgaacactattgctacatgcagccatcagccttggaacaagggaaagcttgtcgggcagaaaaccccgctccgagtcagagatatttgggccatccgggtcaggctccagcttgcggagaagacacgggatctggctctcttcaacctagccatcgacagcaaactgcgtgcctgcgacttaaccaagctgcgagtacgagacatagcccatggggaacatgtgtcgtcacgggccatggtgatgcagcagaaaactcagcactcagtgcaatttgaaatcactgagcaaacccgaacggttctggaggcttggatgcatcaggcccaactccgcagtgaggacttcttgtttccgacccggttgcacgactcagatcatctctccaccaggcaatacgctcgaatagtcaaagcctgggtgacagccattgcccttgacccaactatgtacggtacccacacgctacggcgaaccaaggcatcactgatctatcgcaggacgaagaacctgagagctgtccaactcctgctcggtcatacgaagcttgaaagcaccgtcagatacctgggaatcgaggttgatgatgccctggaaatggcggaacagacggaagtctaaccatccatcgcgacggtcgattctagaccgtcgctatccggccaacagcggacgccagagacggcagattctggccataaacacaggcggcacaggcctccaacgaagatatggttcttttaatccgtgcgcgccatcgccactcatcggtttagatctcgggatcttccatacccctgtacattgtggcacgatcagctgtgacaaaatgccattattacggataaggtgagcgttatgatcaaagggttggatcagttgcaacgcgatttaaaacaggcgcagattgcgcttaaagaactagatggcactctttgtacgattaatttcgatcccttcgatcccgcaagcattgagcatgcaatacaggaagtcagcaacactattgatcagcgcgttggagtttatgctggcaatccctttgtaggacctctaattgaaggcatgaaagaaaattatcgctcgcggataattgagcaggcagccgaaaagcgcctaacaggggaaagcaagtgagctcctctgatatttttactcagattaataattgcgtattggacctgcagtcttcccagcaccaaacatatgcagtgccattgaagaaactagcacgacttttatctagccccgaactcgaatccgtcaatgctaacttaacgcaaaatgcagacctcgaagcttttttatctgaaagcgaagctactggtggaagctttgcaggcagccatcggttagcgtggccagatgacgacgaactcaagcttggcttgactatattgctaatccagaaactttccaccgatccgaactacgcattaaactttggatatcacttcttcagcaatggtagcaagaagatgatttccggccttcacgcttttgtcgctcaagtaattattccgttcgcgagagattataagtctcacgtcaagattagcaatgcagcattggtcaggtctattgttcggtccaataaggtcttcattgtgcacggtcatgatgatggggctaaacatatgctagccaggtttattgacagattaggattagaatcaatcattcttcaagagcaacctgatcgcggcagaactatcatcgaaaaattcgagcagtccgcagaggtcggttacgccgttgtactactaaccccagatgatgtaggcggggctgtaaaggcagatgcgccctcagcacgcgcacggcagaatgtgattttcgagctaggatattttgctggtaagcttggccgaggtcgtgtatgcctcctgagaaaaggcaatgtggagattccatctgaccttttcggcgttgtctacacggagcttgattcgcacgagggatggcaaaagcggcttgttatggagatgaaagaggcgggtttagatttcgacgcttccaggctattctcctgactgtatagcgcgtgggctaaaactagcgaaggcgctggtgcatagctaatatatacgtctttttatcggttgcttctgaacaccttagccatggcggcatagtcgcatttggtcaagggagaacttccaacagctgctgtaaaacaggagcaggctacatttataaccatggaggcctaacccagtttacgtgctcaacttttcaagtgaagctgaaggcctcatcaatcatggaataattatgaattacgttgacactgcatttagacaactttctcttgcgtggaagctatacgactatgcgcttgatggaaaaatcaatttagatgagctagatccccccttgacattccaaggtggcggtatggttctagtgcttccggataaagttttagatactcctgacgacttaatattggctctgcagaacaatttggtcattacatttggcgcggcagcgatcacgcttaaccgttgccgagaagaagcggggtatgcgctttccgctgaaattattactgaaaacgatcagttcatcgcagttacgtatcaaatacgcaacgcgttcgctcacgatattgccgagccacgctggaacattaacagagcccgttatgctaggccctacgaatttggcggaatacacataaacctgacagatgttggcacgaaaagattcgagtatcaagacataggtgggccagacgtacttttcctaatgaagacatatgcagagactcatctctggccttgaggcttattcctatgagcagctatcacccttaaaccaagaaaaaaaagagttcagactaaacttacaaacggtggtctgctcccgatatcgcagatcacatttgcagtgcttgctatctttccatgcaggcgttatttaggtcgcctttgagctttgcttaaatggcagcaaagcatacgctttcggcggaaggtaaccgaccccaaagctgccattggtgcagggcagctaactgcaaatagcagtcatttcctaaattttcgataaggagcctgatttagccggttccgaataggcgaagcgaacggtttgaaccatccaacagcatttgcaaggcttactggggaacacctgcctctttcgcaatttcatgaacggatcgcgctagagactgcttaatttgttgtaagtcgtcattattttttctcccaaatccaataacacaggctgccgcagcatcaacaaaaaaggtacttgcgatacgggtcatcattgtagaataggcccatgcttctttagccatattgaccttttgttcgatgggtatttcaagcgaaataagccacaaaatagtgtcttccccagtgagatggcttgcgccacttaaacgatggtagctttcgtagtaatcggtcttacgccccatcgcttcgaaacgcttaaatagcgactttggccactctgtgcttttatccacaggctcgattaaagcttgcgtctcaacatgacctacatatttttctagagattgaatgaagtcactcctctcatcaatcattgccaaaactttttccgcataactttcatctctgatcgtttccttccactcagaaagttttcgtccgtgctcatgcaaccaagacctaaaaaattgaatcaaagtgctagagtttccgattgtcgctaaatacatgatattcatggctccctctacaactacccttgcgagtgcttcagcgctggcaggggagcctgtagatatggcaaccaacataccttcagagtgctcgtgaatacgcccaagcaggtttatcaaactgtgaattctgaagctttctttagcattggaaagtttaacttcagacaggtactcggtgacaatattatttgtattataaattgcgtcaacagcaatcaatgagttttgaaggtcagcatggggggcgatatggaatttttttcgaaaatcttcaatatgactcacagattaaatcctccaataaaaaatgccaactcgcagtaaatacttgcagttctatgttatccggtgtccgaatcgagcgatggccgggcgtactattggaggtgtccttgtaggcccctgatatagacaaagcgattgcctctccagttaaataagtgcgtctttaaatctcacgaagatacgatgtcgctagcagcatgtctatggcctgttttttggcctgctactgctgcttgcaacgagacatcagcccctttctcaagggaccgcgttgggtcgattgctgcctttcacgtagggctgcaatcggccaaaagcggactctcggtgactccaaggccacgccctattcattctcccctcgcgtaaaaacctacgattggctccgtcccttcttgattcgcccactttcaatagaaaatgcgacgcacctgtagtagcgttgagccatactcgtgaggttgcgcagaaactcggccaactctttacgcactgcttggcaccagtgcaattcctcaatggatgctttgatatcactcaatggactcaaggttaacttatgcaatctctagcggcctatttacttgaacgaactgtaaactctgaagatgaaaaaatatcattaatagccgaaactagaaagcacttaagtaattggcttaaagaaaaaggagttgcagatcctgctggcagttcaggagaattcaaatccataagctcatctgaaaccggccactataagcgcgagaccgcagtaagcaacgatgaaatactggagcaaataagacttgaggagtcgcctagaaacaatcaaatattttttacaaatgtagcgttcgccacatccaaaacaagattttttgtatacattacactttcagccacgaccaaaaccagcattatctcccctatatcaattgatgctcgatgcccatcaattctgcgtgatatcttaagaaacggtactcagtggaaagtaggtaattacctagtgcctcacggtgatcgcgtacaaataaaaggcgatgaaaaaggcctcgaacttgcgcactatttaaagtcaagcacgcgaattttcccagttgtggttgtttccgaatacgaaggagagcaaatttggagagggcttggtcgaaagatcgcccatgaccttgctggcctagctcaaatttacgaagtggatgacaaagcctcttgggctattacagatgtaattgaaaagcaaaactcttgttatagcggcgctataaggctttattggccgagcaatggatccagctcagttgagcagttccatggaaccttgtggacgccatacaaattattatctaatgataaggacggggaagcagaagctagatttcgtagacaaatccgccgacgtgtcatgagcgtatctgcacttactattttgccaccaaaagaaattcatgaaattcagagcgctagtgctcgtaagcggttaaccgatttagaaggtaaagcatcatccaccgacgacttagtggaattggctcaatcatatctcgatgatgccgatacgctccgatctgagaacacagagcttcaagaaaaactatctttagcgataactcgcgcagagaatgcggaagcaatcgctgaaaacatttcaagaccactgcaagagtttgacaccgaagcccccacagaaaatggtgatgatgagcaagaggaacaagacctctctccacccgtgccaggagagataagatactacaagaaagtccgtaacactccttctcatgaccttctaacgcacgtcgctgattgtaagcatacgagttggcaagctgcccacaaagctgaaaaagcgaagaaaggagtggagaaacttgaaggtgtcagcaattgggatgtaatacatcattgcggaacgtgtaaggggggaggaatgtggagagttaaatggtgataatcgccacttgaattgactagccattgtttgacgatcaaagacttgctcaattgcgagtctttgacaacccaagctgtagctagtgaggcccatgagcgctggcttttagggagtagccgcccaatccatcacggtggatgtaagagcgtcttcagtagatgcgagaaacgcatctctcaagtgggccggaatgtcgatgatccacaaatggttgtcctacggagggggctccgtgctcgcgtctcc

SEQ ID NO: 3 - DNA, 16414 bp, unidentified
  source 1..16414: mol_type = unassigned DNA
ttaaaggccccgagcgcttatagccctcggggcctttttcatttgggggaattttgggggaatggggggacgtgtaattcccccaagcgttcgctatcattccgccatggcctactacgagaagcgcggcgacgcctggcgcgcccagatccgccgcaaaggatacccaaccctttccgccaccttcgacaccaaggcagatgcccagcgctgggcagccgaggtcgaaggcgatatgtctcgtgcgcgcttcgtcgacatgcgcgaggccgagagcaccaccctggccgaggcgctgggccgatacctgtccgaggtgacctcgaccaagaagggcgccaagcaggaagaggtccgcatcaagaagtggaaagctcacaagctggccggcaaaggcctggctgctatccgctcaagcgacatggcggcgtatcgcgatgccgagctcaaagaagggaagtcgactgccacggttcgactcaacttggcggtgataagtcacctctacacggtggccaccaaggagtggggtatcgaaggactgaccaacccatgccgggcgatccggatgccaaagggcagcaaggagagggatcggcgaccgacgcctgcggagctcacagctctctacaaagtcgcgggaaatatgaatgcccagttgccggtgttcatcgagttggcggttgagacggcaatgcgccgttctgaattgctgctgctgcgccgcaaccaggtgcgaggcaaggttgcctatctggaagacaccaagaacggagagcgccgtgcggtacctctttcttcgcgggcaatcaccctgctcgaggggctgcccacgccgatcaatggtgggcggtacttcagcctggcactcaacacgatcagcaattacttccccagggcttgcgtggccgctggtattgaaggcctacgccttcacgacctccgccatgaggcgacgagtcgattctttgagcgcggattcactatgatggaggtgagctcaatcaccggccataaaaccttaactatgttgaaacgctacactcacctgagtcctcatgatttagctgaaaaaatgggttgaaacatcggttttaatttttgttgttagttgtcaaggaatgataagtggttttcgaacaggagaggaaaaatgattcttaagtcagttgaatattatgagggtagtaagacaccgcagttttgggcgttagataggcttgacctaggtaagaggaatttggttgtaggcaaaaactctactggtaagacgcgcgctttaaacgtgatagttggattggcgagaattatttctactgctggaagtttgcctgattcggcaagatatgatgccacttgggaggataagagtggtaaggtttttcgatatcaactctctctcgagtcgagctcggtacagtcggaagttctttcaatcgatggacaggttgttttggatcgctcggctgggggggtaggtcgaatatgggctgagcaagtttctaacggttcaataattccttttcaaacacctaccaatgagctgtctgtactaaagcgccgggattctttgcagcacggctttatagagccattatataaatgggcttcgcaggttcgtcattacaacttcggttctagtttagggaaagatcatcttacatttatttctccatctgcacctgccgtagatgaaaaagatcagaatcaggttgtaggtatttttagaaaggggaagaaagagtttggcgctgattttataaatgctatcaagtccgatatggcgcgtattggttatccgttagatgatgtgacgacaggagcaccttacactgtgagagttgaaaacgctccaggtgaggttgcttccatactagttcgcgaaacaggtcttatgggagtaactgatagcttcggcatgtcccaagggatgtatcgagtgttagctttagttattcatatgaattacctgcaatttaatcgtgttagtacctgtgtagtcgtcgacgatgtgggtgagggtctggattatgaaagatcctgcgatatcattcatctgctgcgagaaaaatcggaagcctcagacctgcaaattataatgtcaaccaacgatcgtttcgttatgaacgaggttcccctgcaagagtggactgtgcttcatcgatatggtgcgaaggttgaggttagtaactatgggaattccaaagatctgtttgatgacttcaagttcacagggttaagcaatttttccttctttgaaatggattttttaaaagaatctcgcggagattgatatgcgacggattgctttttttgtagagggctactcggaattattatttgtagataagcttcttgtggaaattgccggggcacataatgtcgctatcgagcaaaggcagattagtggtggagttagggttccacgttctgtcaaggtaatccaggcggctaatattgatgctggccaacaatattatgtgcttatcgtggattgtggaggggagtcgcaagtgaagacacgacttcaggaggagcatgaggggcttactaggcaagggtacgaaaaaataatctgtatccgggatgttcgtcctgagtttactcgagaggaaattcctaggctagagcgagggatgcgcttgtatgtaaaagggagtcttgctccggtagactttatcttgactacgatggagctagaagcttggtttttggcggagttcaatcactacccaaaaattgacccggcattaaactctgaagctgttcacgagcttcttggataccatcctgaaacagatgatcctgggactcgagactgccccgctgacgatttgcggtcatgctacgctattgctggaaagacatacgaaaaatcagaagcaatccggacggtggaagctctggactatttatatgtttataccgacctgaaggatagaattcccgaagtgggccgaatagttgcccacgtcgatgagtttttaacaccttcatcctgatggttctgtctaagctacgcctttcactgaaggtggagggcggcgggttctccctacctttggcttctgctgacccgcatcccgaaactcgcgcagaaacttgcgcacgtcctccttcagccagcaatgccggttgcccatcttgaagcttttgggcagccatggcactccgcggcgaatcccttctctgattgacgcctcggtccgaccaagcagcttggccagaccctcgaccgtgagcacttccgtttcttcgctcattccttcctcccggcctgacacgtcaggttctcgccttctcgccgacctgtcgcgtcagttgcctgtagttccgcgatcaccgacttgatgcctgccacataactgccagggcgatcgaccgccgcacctgtcaggcgctcgatcacaacctctaccggcgaccctcggagcgagccgactaggtcaatcgcccagttgcgcccctccaggaacatgaagtggttaatcgggccatccaccacgatctcggcactggtcttggtagcgctgacggaagtgatcttcgcaggcgccttggcggaagctctggactgcactgagttaaaccgcccacgagcgcggcagagcgccatatcagctacggtccgcatggctggcgccctccatttcggcgacggcgcgcagacgtagcgtaatgccgcattcccttgccaactggtcaagccttccaacgctggtggtgctgtcctgcagcgcctggccgaagcgcaccagccgccggcccaggtcgtcaaactcattgcgaggcttgatggcctggttcatggctgctgcacctgcagttgttccaggcgtatggctgtgtcgatctcctgatccagctcagcgccggtgaacagggtgtcgccgcgcagcaccagcagatctgtctcggcgtcctcgatacactcccggtcacgcagccaccggtaccgcttggcatcagccatcagcttgacgtgctcatcaatgtcgaactcggaagtgttcgctggcgccaaccggccagccagcaccagcgcgccaagcagcacttgcttctgctgctggccgtgcaggtactcgcgcatgcccttgatgaaaatgctgttcatcgagcggtcatcggcatcagctgcagcctgaatatcgtcacgcataccgtcgggcaggcgaacaacgaatttgtcagcggttcttgagtcgtagttgttcacgatctatctcctaaaagcggggtggtgatcaacaccaccccggtgggactacttgcccacgccgatgaatggggtcgcggtgccgctggtcatgtacaccggcaacttcccgtcccacttctcgatcgcattgagctcaactacacctgggttcttgcgcagtgcctcaccacgaatgttcagcgactcggcttcgccttgagcgcgcagcaccgcagcgtccttcaagcctttcgcttcctcgcgcgccttgtcggcctcagcgatgacctgggctacttcgttctggcgctgggccgtcttctgggttgcctcgatcttcaggttcagtgcggccaccactttttcaggcaggccgatctcaccgttcaggtaaaggctttcaacaacgatgcctttgccgtcgaagtggtcgcgcacgcgggcctctacgtccttcaggaagcgctccttgttcgggccgtagatctcttcagctgtgagcttcgatgcggtgttgttgaaggcggtgcggatcacctgcggcacgttgacctggacgatctcatccatcgacttgcggtaggtctggaacaacagcggcgcggagccaggcttggcgcgcagcgtcattccgatcggtgtgctgatcttcatgccgtccttgtcttggaacgtcacgacaccgatgttgatgttctggttgaaggtcgggaacaggaacaactcctcgttccaggtcagccacttgtagcccacgctggtctcggtgggagctacacccttgtcgctacccatcaggttgacgatcacccccgtgtagccggcgggtaccttggaacagcctgcggtgatggcgagcaggcacagcattgcagcagcggcgatccgcttcataggtcttcctctttggtggttgccgcaggagcgcggcgcttgatgaaaaggtgggcgaacaaggagatcgaggcgatcagccaggcgccgatgagggtgaagccgagcacaacctgaatatccgactcgctactgatgaggcctggcgcaatgaagcgcaggaccgccagcgacagggccaggtagagcagggcgccagtcagcgtgatcagcaggtcaaacgttctgatggaggggtctttcatcactttctccagggcgagcaaaggcccgccgcgttgttggctttcgcgaaaaatcagggttgggttaagtcagtagggcgccgttacgccaccgcccaggcgctctcggcgcggcggtgaatacggagctcgacaagcttgcgttcaccggggcggcggacgcgggtgaattcatcggtgccagcaaaggagtgcccggccaggatggcgcacaaggtgatgatcatcggcgagataagaccgagacgcatggcctcggccacgagttgggcgcgcttgataacgccgagcttggtgctggcggcgagcagacgtttatcgacggtgtctttggccacgccgaactcgcgggcggcttccttgctagtcagtccgcaggccaccgccatgacgcactgcagctctcgttccgccaggcccatgcccagatggccggtccagttttcgaaggtcagtgcgttcatgtgcgtagctccatgcggggtgcgatggggcaagattacaactagcatttgtagactgcaaatattatttgtaaatcgaggcgcaaaaaaaccaggcaaggcctggtttctgttgaggctaaccggctaccagagaacggatgaccagaagaccttgccaagaatgacaatctcgttgtcgatcatttcttgagcactgtactcctcgtcaggatgatcgtcgcgattgaagctacgcattcggatgccgccgccgggtaagcgataaagcgttttgacgcggagctgcccgccatgattcagggcatacatcttgccatccacaacagttgttgcaccccgatcaaccccgacagtgctgccgtcggggagcactggctccatgctgttgccgctgacggacacgcacacagcctcactaggctggaccccttgccggcggagagtgagctttccaaagcgaagctttttctggggagactgctctacaacggttatgccgctgccagccgatagctccacttccttgaggaatggcacatagacctcgtcttcatctaggggggtactgtcatcccagacgtcgaaagatccgacgacttttgcgtttgagtggacgccctgcctagctgtgtcaacaagcccccgcagatcttcggatttcactacgccatctttattgagccccagaatggcaacgctcaacaggctctcaagggagatgttaagggtctctgcaatatcggcatacatgagcgcgcgcggtgtggatcgacccgactcccaagcctgcacagactgcggcgtgatcttgagtcggcgcgcaagctccgactggctaatgccagccgctgtccgcccctgcttgatgatttcggcaatagtcttcatggggcaagagtacaacctcgtgttgtagatttcattgcaaattagatttgtaaaaaacagtttgcagttgtaggcttttccgcaatgtcataaatccgcagggtcgaccatgagtaccgaagctatggcttcagccgtaaaggcggttggaagccagactgccctggcaagagccctgggctgcacccctcagaatgttcagcgcatgtgcgcaacaggcaacgttccggcaaaacatgtattgcggatagaggccgcctctggcgtatctcgttttgcgttgcgcccggatctctatccagagtcattgccgaccctggaccaaacgataccggcatttagccatcggaagcagtccgatgaatctgctgtaaatccatccagtacagcgcgggcgaactcatgaaacagtccatcgagctttaccgccagtgcaccgttaagcccctcgcgctccggataccggcgaaccgtcacatttgggatttctttaaaccagattaaaagtcttctcagcagctcgagcagagcatgtgacttgcaatttttggagccgtgatatgcgcacgcgatctttcattccgccgacccgtccagggtaggccacgcccctctcaagagaggggttgcatattttttgttccgtggatgattgggattagccaaatccaaggcaacaaaaaacccgcttgccggcgggtttcttaatccactccttgccgggagtggcttgtacttcatcgcttgaaggagcgagaaaatgtcacacccagaaaatagcacccagctatctaatccgcaagacacccactcggatatcagggggatcatctacctcatggtctgtgcagataccgaggatatctcgtaccaatgggagccgttcctgcagaaaggactggccatcgaacttcttgagatgctggcgccagagtttccgggagcacggatgcgtttgatccagtgcgccggacttgtttcggatcttgaatccgttttgggggcggctgagcgccagaaggacttgatcattagttgccggaacgccatgcgacctggccgcacataccttgagcgaatggccgcgaagcgaatcccaatgcccgcgccacaaaacctaacctctcaagttcgtggcgcggaggttacccaatgccaaggccaatgagcgacttttccgcgcctacccggcggatcgaagaaagtctcgagctgctgggcgttctcgctgaagtgcttgagcacaacggtggcttcaagtacgacgagccaggcgagcatccatcaatgatcggtgatcgcggagaggacgggattgtccgctcaatgcgggtgattgcaagagccgcccacgctgaactgtgcaggctggcaaccgacttggagatcccccaatgaaccaagttatcccaacgcggcagtctgccggccttcaaggcgagatcgtgcaggacgtgatcctctcggccgaggaaatcgcacgcttcaacgaagcccgcgaggccttcaggatgatcaaagccttgtactgggcgcagattgtccccgggctcggtggcttcgacaatcccgtggtaggcgagcttgagcgccagctggaagtgatcgtctttgccacgcgcaactttctgtacccccaccgctacgcggctgccttccgtgaagcgaaagatgtgggaggtgcagcatgaacccgatctgcaataccgccgtgcctacatctcacccggccctccaaggcttggatcagggccagctgtccgagcttgctctcatgggccttcgatacaaagccctgggtgctggcgcaattgacttcaacgacccgtccaggctggacgtttattggactggaaatcgaatggttgagcagagcgtcgaggaggccgtgaaggcctcaaagtcccgagcagtcaatgcgagttacaaggccgggattgcgactggccacttaatggccctgttcaactgcagcgttatcgacaacgccttttacatggcgcagttcggactgctgctgcccaaaagtgcagggggtgctgcatgaacctgatcaacacaaatgccctgaccatgtcctcgcgggagatcgccgatttggtgggctctcgccatgacaaggtgaagcagtcgatagagcgcctcgcagagcgcggcgtaatcgtccaacccccaatgggggatgaacaatctcccgactctttggggcggcctcgcaccgagtctgtctattacgtcatcaagcgcgacagcttcgtcgtggtcgcgcagctctcgccggagttcaccgcagctcttgtcgatcgctggcaagaactagagaaccaggcaggtcgcccgatgacgcaggccgagatcaccgcggccaatgccaaccacttggtggaggttgagcgccagcagcgggagcagcaggcagcgctggcgaggatcgagcgtcgcgtcgacgacctgagccagaccacggtctgggatcactgcccgcagaactgccagtcactgacgcgcatcaaggaaaccatgctcaagcggcatggcttatccggcgctgtcgtggactacgtgctcaaggtctggccgaaccagccaaacccggccggcatggtccgcaatggtcacgaggaagcgctggggtcgcagtacctggtctggtcaaagagccacgtcacggctgccttccaccgatttgtttccgaatccacgatggtcactgccactcaggcaactcacccctattttgagggccggttccgtctggtccggaaggtagcgccatgagcaaaacgatgaataccccgggccagcctcaagtaatcgacacggcgcattttcagcagttctctgatgcggccctactcctgatgtgctttgagaaagtgatggatgcaatagggttggtcgacgaaggcgtcaagatccgcgagtttgacgagacctatgtaggcctgattgaggcgaccctggcgctgggggtgctattcgagcgccgcaccggccatgacgcgacgaaagtgtcggctgatcacctggaagaacaacgccgccgcctactggcaggcgaggaactgaaatccttgtttatcccggtggtaggtcccggtatggcgccgttgcctgcttcggcattctctggcctgactaacttggaactggccagcgcagggttcaactatgccgatagggtgcgcctggcgatcgcgggcgattcgctcagagaagtagagttggcggatgcgcgagttcactcagtcgatgccattacagcattgagcaccctggtcatgcgtcttgctggcggctctatggccgacctggccaagcacgcctccaagatcaccgggcctggctcggagaccctgcaatgaacaagccgttcacccctacccaggcgccacagcagcgcgctggcgccacgaccattgccgggccctggccgagctattcgcagttcaagggcctgccagagcgcgagcgctggacgctgtacgaactggccaaggccggacgactggcaatggaagataaaggcttccagatggccgagagttacgacgcctttgtgcgcagagttacagaggagcttgacttgtgacccaggaacgcattccacgcaaattccaaggcgtttggatacctgcctcgctgtggttggaccattcgctgtcctcgaatgagaaggtcatgctggtggaaatcggcagccttgaagacgacgtgcgcggctgttacgccaccaacgcacacttcgctggcttcttcggcctttcgatctctcgggtgtccgagtgtagtggtcaactaatcccggacactgcgttaagtttctcctcggccacagcgggcgccagcccgcggttaaattgatgtggccgttgccagttgtagcgctgcatcaaaaaccgaccaatatcctgctgtgccagcgaagcactcatgtagcctacggttggcacccattctgttttcagactgcgaaacaacctttccatcggcgcattgtcgtggcagtttccgcgccgactcatgctctgtgtgaagcgataacgccacagtcgctggcggaagcttcggctgccgtattggctgccttgatcgctgtgaaacagcacactctgtggccgaccacgctgttcataggccatgtccaaggccttgatcaccaagtcggcatcgggcttcgatgaaaacgcccagcccaccacgcggcgggcgaacagatcaatcacagccgccaaatagtgccagcgaccttgagcccagacatacgtgatgtcaccacaccagacctcattgggtgccgatacgctgaacgctcgatccagcacgttcggaatatccggccgctcgaccgtcgcctttttgtaggcatgtgagccgggttgcttgctgatcaacttcatttcgctcatcagcttgcgcaccttgaaacgcccgatttctatgccgtcctcgcgcatcatgaacatgatgcttcgactgcctgcggcactgcggctttgggtgaacaattcgtttacacggctgcgtaaaaccagccgctcaacgtcgggagttcgacgttttcgacagtgtgcgtagtagcaagatcgggtgacttcaaataccgagcacaacagatcaacaggctcctcagaacggagttgatcgattaacgcgaacgctcgtgttcctcggccatcaagagcgcggtggccttttttaatatagatttttcccgttccagccgattgatccgagcttccagctcctggattttttgctgctcgggcgtgagcgccttactggtcggagtgacaccgcctcgttcttgctggagctggttgacccagcggcgcagggcagactcaaccaaccctagtgagcgagctgcttcgatatggctgtagccctgatcgagcaccaggctggcggcttctcgcttgaactcgggcgtaaaggtacggcgttgcttggtcatcagacacctctctgtggcgagcattctcgcctaaatgggtgtccggaatcattagaccactacagagatcatcagtgggctggctgggcggggcctgatcaaggtcgagcagatccgcgaaggcaagcgcgtcattgagcggcgaatccgcctttctaaccccttcgataaaccgaagaccccttcggaaaacgccgcgaaccccttcggaaaaggcgcagaacccccttcggaaaacacgcaggggagtaatacatctcagagtaatacaaggagtaataaagacttacgtgcaacaggcacagaagcggatgacgggttcgagaagttctggaagctgtacccgaagaagaagagccggaaggacgccctgaaagcctggaacaagctgaacccaggcgccgagctgcagacggagatgatcacagcgctggggaagcattgtgtttcgcgggattggaccaaggacggcggccagtacatcccgatggcctccacctggctcaacggcgaacgttggtacgacgttctgcagccagctggcgcagtcgcccagggcagcgcgttcaacaacctcccgcatcacaccgacgacatgtaccaggagagccacgatggccgctcgaatttctgatctgttccaccgcaccccggccaaacgcatcttctccggtgagtgctcggtgcatggccgcgtcgacatgagcgaggtcgagcagttggatggctcgatgctggcgcgcggctgcaagcgctgtgcctgggaggctctgcacacctcgccgcgggattcggcagagcatgctctggccagcgcccagcgcaagaccgaggaaaccatggccgcgctgatcggcgccgggatcactccgcgattcgctggcgcgaccttcgactcattccgcattggggctggtagttcccaggtccacgcgctggaagcctgccgtgtttacgctaagcagtttccccagaacttccgcgccggccgctccctgctgctgaccggtaacgtcggctgcggcaagacccacctggccagcgccattgtgcgcacagtggttgccgatcactgccgcgcgctgatcatcccggccggcgatatcgtcagcatcgctcgagcttcgatggtgccgggttcggggtacaccgaccgcgacgtggtgttgcacctgggcggccttgatctgctggtcattgatgaggtcgggtgccagaagggcagcgagtacgagctgggcctgttgcataacatcatcgaccgccggtatcaggctgtactgcccaccgtcctgatcagcaacctcgggcccgatggcctgaaggcctacatcggcgatcgcgcgcttgaccggctacggcagaacggcggtgagctcgttggcttcacctggtcctcgatgagggcctgcgcatgagggagatgtttagcatcgaggctgagcacggcgtcttgggggcggtaatgcaggcctccctgcagcaggacgccggcttggttgaggacattctcggccaaatggaatcgggcgacttctaccacgccgacaacgcggcgctgttcgaggtgatcctgggtatccatgaccagggtgtgccggttgacccagtcaccataggctcgattcagcgttctctgcccagcggccagctcaccatggcctacgcggccgagattacgaacaacgtgccgtcgatagccaactggcggacctacgccaagcatgtcaaggaatggggggtgatccgccgcattctggacatcgcgggccaagcgcaggagctggtgcagagcggtgcgccaactgccgaggtgatcgccgcctcgcagcaggccatggccgatctgcgcagtcttgacggagaggcgaagggcttcaagcgactggatcagtggatgggggatgccgccgatctggtggacgagaagcatcgcggtgttgcacccaagtggccatcgacagggctggctgatctggacgacctgatgcagggcattcggccaaagaaagtcacggtcgttgccggcttgcctggtagcggcaagaccacgctggcgctgcagattgctcagcacaacgcgatcaaggagcgtaagccctggctggtgttctccatcgagatgccgggtgaagagcttgggcttcgggctatcgcgtcgttgggcggtgtggaactgcgcaagttggacgatccagtgaagatgcgggatgaggactggtcaaggatgtctggcgccgtggccattgcgcttgaggcgccgctgttcgtctgcgatgagccagttcagaccccggccagcatccgcgcgaccgccaggcgctgccagcgtgagcacgggcttgccggcatcgtggtcgattacttgggcttggtgcgcagcgagcgccaaggccgcacccgaagcgaggaagtcggaaagatcagcaaggcgctgctgcagctggccaaggagatggggattcccgttatcgaactggcccagctcaaccgcgactcgaccaagcgccccgggaagaagccccagtcgagcgacctgcgcgactctggtgagatcgaggccgacgccagctgcatcctgatggttcaccgcgacatggacacggaggaggggcagaacggcctaaccgagatcctgatgaccaagtgccgacatgcccgcgtgggtagctgcgtgctccagcaggagggccagtacggccgattttccaactttgcaggcaaccgcatgcccaccgacgatgaagtcgagatggcgcggggcagctatgccagccgctacaagggagacaaaacccatgggtaacgtaactgcggccctgccgcgcaagagcttgaccgatgttgagcgcaagttcctcaaggtcggcaaccggatgctgctggagcagaccaacggccgtattgcctcggcagcgctgatggacatcgtcgccgactggcacggcaccagggcaagtatcggattcgagcaattcgcaaagagctggatcgccgaaggcaacgccaagaacaaacatgccaacaagctactacgagagctgttcggccttgaccaagatccgaccccgcggagggctgcatgaagaaacgaacctacctggacaaacccctgggcgacaccgagtacctgctggagcaatggggctggtggcggatggatggtatgggtgtgcctcggtacgtctccccgctgttcgccttgatgcgcgacaacgtgccgtctgaaggcggcatgaagcagtacatggtgactgatgacctggcgctgataatcgatggcgcggtggctcgtttgaccaagcgaaaccagcagatgggcgactttatttggctctacttcggggcgaagcagcctgcaatgcgtgttggaagtggggcgggcatgtcggaacgtaaggccagagaaatcatcaaggcgggtgtcgcctggattgattgcgcgctggaagaaattcgagaggctgcgtgaaaaacttctatgcgggcggataaacacctgctttcatagcagcgtgtccagcttgcaacgcatcacgacactgagagccccggcattgagtcggggtttttcttttttcacgttgctgtgtctagaatctttctgcggacatgtttggtgtcgctcacttgagggaataaacgtgaagagatgtttgcattttagcgcggcgctactgatttaccttgaggacactcttgatcctctcggggccgatagttacgacttactcaattacttttcagatcagctcaacgctgaagaagaaaacgagcaagccctccttcaagatcgcctcagctaccaccttgcaatcctcgaaggggccgccttgatccgggggcaaacccaggagggtgacgaatcgctttattacaccctgacgtgggcgggccatgactaccttgatgctcatagatctgatgcgcctaggagctacgcaggcttgctctgagtaaggttctgatatttgcccagtcataatgctgggctttttgtttttgcagatgacgcgcccaggcagctgggctaagtcggtagtggcgtcgatcaaagccgtgcgctccctgatcggctacgcgatgagaggctggggtacgtgacccagcgatccagcccatcaagccgggtaagcaccggccctctgcacccattcgagcctcggcacctgccggggcttttttgttccaggagcatgaagatgagtgaccagtcacggtttctgactgcaggcaaactttcgagtatctccggccaggtcgatatcgacctcaagaccggggcgttcaccatcaaaggtccgcctggcagcgtggtcatcggcgacatggagaagggcgacgttgttgcccgaatcgatgccgagcctaccgtcgagccgttgcgccttggcggggtcacgctctacggtgagctggcccgtaacctgcgcgacgtgcaggcgatgctggctgcccacggtgctggtgagttgaaggtggtcaagcccggcggcgagcccggcaagcccttcttcatcatcgacggccgagtcttcatcagccaggccgaagtcgacgccggcaagctcgcagtcgaatacaccatcaaggctgatgctgcggacatcggccgggaatttatggccggcctggccagttgcagtctcattgatgcccgggtgttcaaggtcaccgatccagctgacgccatccgccaagtcatccgcgaagagctgcgaccaggcggcatgctgaactcccgctaatcctgctgcacctt

SEQ ID NO: 4 - DNA, 14940 bp, unidentified
  source 1..14940: mol_type = unassigned DNA
gtctcgcaaagcgcaagggtgaccccatgatcacgctgactgacgtcaaccgccgccagcactatctggctccagccgccattgcccgcgtgcaggaggccggcaccagctcgcagtggtacggcatctgcgccatcgtccacacgttcgacggccaggtgctggaggtgcgtgaacgcgctgccgatatcgcgcagcaactcaacatgcgtaggactgagtgatggcctgcagcggatgcgccggccggcgcgaatggatcaacaaatggacaaaggtggcatatgagcgagccaagcaaatcattgtcggtggcgacgatcgtaccggcagtaaagagccatccggacaatccccaccccgtaatggggaccaaggttctgctgagtgacggtagcgagctgaatggcgtgacgagtgtggagctcaaggcttcggtcgagggtggtgtgtggcatgcagttatcactgtcttgccgcgcgagatcccgactatctgcgccaacgcacggttcgttgaggtggatatctccgacctcaagagcactgcccgcgaacacgctcgggtggcgccatgagcatgcggcaggtgtcgttgctggagcggatgctggccgaacaggtgaagcagaccgagctgctgcagcagatcgcaaagaaccaggtggtactgatccaggctctggccgatgagcaggatgtggatgccgaagaattgcagcagacctacctgagcggccagccatgccgatgaggcctcagcgcccatgtcgcgcatcaggctgccgggcccttcaccgcaatgccaatggctactgtgatgctcacgccgaccaggtgaagagctttgtcagggagagaccgcgagagagctcgaccgctcgtggttatggctacaagtggcagcaggcccgtgctggcttccttgccaagcatccactgtgtcgacactgccaggccaaaggcttggtagtggtggccaccgatgtcgaccacatcgtcccgcacaagggcgatatgtccgtgttctgggatcgttcgaactggcagagcctatgcgcaccgtgccactcggccaagactgctgccgaggacggtggcttcggcaacgcgcggcgctgatcgtccgaaacgcaccaaaacgggcgaaatgagccgcaatcggcccgcaagggaggggagggtcgaaagtctgggccttttcgcttctagaccgcgccctcagtcgtttttttacacccgcgaaatataaagtttagtggaggcgccgatgccaggggttgccgggcgctccggccgtcgcccaaaacccacggcccagaaggcgttggccggcaatcccggcaagcgcaagctgaacaaggacgagccagatttcgccctggtgaccaacgtcgacgcgcccgaatggctgtgcgaacacgcgaccagggtttgggaaatgctggttccggaattgctccgggcaaaggttcttgccctgaccgacatgcacaacgtcgaggctttctgctctgcctacggaaactggcgaagggcgcaagaatcggttatcgcccacggcatcgtggtggctggagccactggcgggccggtgaaaaatccggctctgactgcagctaacgaagcgatgcgccagatggtcaccttcggttcgatgctgggtctggacccggccagccgcacgcggatcatcggcggcaacaagcagaaatccaccaacgagttcgcagccctactgagttcctgatggccagagccaagtacaccaacgtcgacaagtcgatggcgtgggcaaagtccgtcctcaaaggaaagtttcccgcttgccgcttcatccaccaggcgatcgagcggcacttcgatgacgtagcgtccagccgatcgaaggactacccgtacaagttcgacctggctaaggccgaaaagaagctgcgcctcatgcagctactgccccacacgaagggcgaatgggcgtccaagcgacagctgatcaccctggagccctggcagctcttcggcctggcttgcaccttcggctgggtccggaagaagggtgggtaccggcgcttccgcgaaagctactgggaagtgccgcgcaagaacggtaagtcggtgatcgctgccggcgtgggcattagcatgttcgttgccgacaatgagttcggtgccgaggtctactccggcgctacgaccgaggtgcaggcgtgggaggtattccggcctgctcggctgatggtcagccgctcgcccatgctgattgaggctgcgggaatcgaggtaaacgcctcgaacatgaatatcccgtccaacggcagccgcttcgagccattgatcggcaatcctggcgatggcgcttcaccttcgtgcgcgattgtcgacgaataccacgagcacgccactgctgcccagtacgacacgatgatcaccggcatgggcgcccgcaggcagccgctgatgttcatcatcaccaccgccggtgcggacattgagggcccttgttacgacaagcgccgccaggtcatcgagatgctgaatggcaccgtacccgacgacgaattgttcggctacatctggaccctggacgagggtgacgactggacagaccccaagaacttggccaaggccaatccctgcatgggggtatcggtgttccaggagtacctggagagccagctggccagggccatccgctcggcacgcttcaccaatactttcaagaccaagcacctgaacctgtgggtgaccgcgaaatctggctttttcaatatgcagagctggaaggcctgcgaggacaagacgctctctctcgagcagttcgaagggcaggagtggattgctggattcgacctggcgcgcaagctggatatgaactcccgggccaggctgttttggcgacagatcgacgggaagatccactactacagcgtcgggccagcgttctgggtgccggaagacaccgccaatgacgtggacaacaagcgcatgactgagcgcttccaggcttgggtcaacaccggccacctgcacacgacacccggcgccgaagtggattaccgggaaatactcgaggacaccaaggaagccaacaagctggctccgatctcagagagcccgattgacccacacggcgcgacgggtctcagccacgacctggacgatgaagggttcaacccgatcaccgtcacccagaactacaccaacatgtccgaccccatgaaggagctggaagcggcgatcgaggcgggccggttccaccatgacggcaatccgatcatgacctggtgtattggcaacgtgatcggcaagaacctgcccggaaacgacgacgtagtgcgcccgatcaagcagggcgatgacaacaagattgacggcgctgtggcactgatcatggctatcggttcggtgctgcgattggtggccgagggcaccggtggattcgacaacttcttcgccaaccccatcgtgcttggctgacaggaaccctatgaaaactggtctcatcatctttctggcgctcgccaccagcggcttactgctgggtgtagcgggtgtgtatgtgctcgcaggtctcggctacggactgctgactgcggcagtcggctttttggctgcggccggatttattcgtaaggggctgacaggtggctaaatctttctcgcaagtgctcggccaagcgatggtcaagtccgccgagcctggtattgcgtcgaacctcgcgggatgggcgggcaagcgtattggcctgaatgattcgcctttctggagtaagttctacggaactgactctgcgtcggggaaggtggtcagtcagcagacagccctccagctgtctacggtgtgggcatgcgtgaggctcatcgccgagaccatcgcgacgctaccgatcgcgctctacgaggacaagaacggggcgccagaggtggccagttctcacccggtcaacttcgttatcagccagcagccaaacgctgaccagacgccggtggagttctgggagaacgtgatggcgagcctgctgctgcagggcaacgccttttgcgaaccgcacatgagtggcagggcgctgaccagtctggagtttttgctaccgcagaacatgtcgccaccgcgccgcttggccgatggcagcatcgagtaccgattcatcgacagcttcggcaagccacacacgctgacggacgaacaaatggtccacgtccgcgcattcggtaccgaccccctatgcggcctgtctccgctctcgtacgggcgccaggtgctggggtcggcgatggccgctgacgagtcagcagcgaagatgtttgccaacggtatgaagctgggcggggttctttcaactgaccagatcctcaatccgaaacagcgcggcgagttgcgggacgacatggtcaagcagtacgaaggcgtgaccaacactggcaagaccatgcttctcgaagcgggtatgaagtatcagcaggtgtcgatgacgccggaagacgctcagatgctccagacccgcgctttcaacgtcgaggagatttgccggtggttccgtgtgccgccttggatggttggccacacgcagaactccaccagctggggcaccggcatggagcagcagatgattggcttcctgtccttcactctgctgccctggatcaagcgcatcgaaatgtgtgcgaaccggcgcctgctgcgccctgatgagcgtcgtcgcttctacgttaagttcaaccccgaaggcctgctgcgcatggatagcgccgcgcgcgccgccttctacagctccatgacgcagaacggcatctacaccagtgacgactgccggatcaaagagaacctgcccccggtaggtggcaacgcttcaaagctcagggtgcaatccaacatgctgccgatcgacaagttgggcgaagaccccggcggcgccaaccaggccaaggccgcattgctcgactggctcaacgaccagccaagaggtaaatctgaatgaaatctgcccccaacagctggtggtctgggcccgactcgaatgctggacacaaggatcgagcagtagcggtcaagtaccgctccttcgactatgacgtgaagtctgtcggcgatgacggccttttttctggctacggctcggtgttcggagttgtcgacagctacaacgaagtggtcgcgccaggcgcgttcctcgagtcgatcgcagaagcaaaatccaaaggccgcacctttcctgtgttgtggcagcaccgcaccggcgagccgatcggtagctggaatatcgacagcctgaaagaagacgaccgcggcttattcggcgagggccagctctggctagcagacgcgccgtatgcccgcatcgcgcagcgcggcatggaaagccgctctatcaccggcctttcaatcggctactacattcgcgagtccagtttcgacgagaagacccgcgtccgcaccttgacgaagctggacttgatcgagatctccatcgtcaccgtgccggccaacgacgaagcgcgaaccgacaccattaagtcgaagcttgcccacggcggcctgccttcgatgcctgaattcgagttgctcctgcgcgaggcaggattctcgaaaagccagtctgcggtgattgccaatcgcgggctgcagcacctgctccggagcgagtccgcgggcgacctggcagaaatcgaactcgtcgaggcgattaaatcgcgcccggcactgtctctcccatcgttttgaggattcaccatgcataacgccatgagcaaccaggctcgctccgaacaacgcactttccagcgcaaggagcatgctgacgacaagatccagctgaaggctgttaatgatctgcttgacgagcgtgatcaagagatcaaggcctttgccagcaaggcggccgccgagatcaaagaacacggcaccatcctgaccgagacgaagaccattctggacggcctggtgaaggacggccttggcctgcaggaccgcctgcaggaaatcgagcagaagatggcgcgccgcttcgctgccaacgaccctactgaagcgaagtcggttggcgaagagctttccgaaagcgaggacttccagtcccttcagacccgtggacgcggtatcgcccggatcggccgcaaggcggttaccaacatcaccagcgctactactggcaccggtggcgtcggtgtagcgatccagccaacccgcatgcctggcatcatcaccgagcctgagcgtcagttcaccatccgtgacctgatcatgcctggccgcacttcgtccaatgccatcgagtatgtgcgtgaaagcggcttccagaacatggcagcagcacaggccggcgagggcgccctgaaggctcagtcggacctttccttcgaactgaagagcacaccggtacggaccatcgctcactggttcaaggcttccaagcaggtgctgtcggacattccgctcctgcagagctacatcaacggccgcgccatctatggcctgaagtacaaggaagaagagcagattctggctggcgacggcaccggccagaacttgcttggcctgatcccccaggccactgctttcaacaatgccctgcgcaaggctggcgataccaagatcgataccctgcgccgcgccattctgcaggttcgcatcgctgaataccgagcctcggccattgccctgaacccggttgactgggctgatatcgaactgaccaaggacgccaacggttcctacatctgggtgaacgtacaagaaggcggcgtacagcgcctctggaagcttccggtggtggacagcaacgccgttccagaaggcgagttcctggtcggtgcgatgaacatcgccgcccaggtgttcgaccgcgaggaggcggctgttgaggtttccaccgaagacggcgacaacttccgcaccaacatggtcaccatccgcgccgaagagcgcctggcgctggcggtgtaccgcgaagagtcgttcgttcacggcgaattcgacgccccgtaaccatcaccggagcgcgcctcggcaacggggcgcggcagaccatgccagaagtcagcgtaaaaaccatcaagggtttcaacaacgacggcgtctacgcgaagcgcggttcgtccattacggtggacgagcagcgcgcccgtgacctgttgcgcaacggcctcatcgaggaatacgacgtgaagaaagccgaagagccagaaaacaagaaggcgccggaaccggctaacaagggcggcaagggcgcggccaccaagcccaaggagtgatccatgcccgtgatcgccatcgacattgccatgcatcacttgcgcgcagaatctgacgaccaggtgctggtccaggcgcaactggaagcggcggaagaggcggcaatgcggttcctcaatcgccgtttctacttggatcaggtagccctcgacgaggccagggctggcgtgtcacaagcgatgcaggatgccaaggcggccaacgcggcggctgttgccgctgccgaggccgagcaggatcacgctcttcgctgccggctgctcgagcatgcgcgacaggcgctggccgaagcctatgaccaggccgacaccatcgcctatggcatggtgctcaacccggcaatccaagctgcctgcctgctcaagctgggccacctgttcgctaaccgcgaggaggtggtgaccggcaccatcgccaccgagcttccgctggcttcacagcacctattgatgccttaccgcatccggatgggtgtgtgatgcgagccggaccattacgccatcgttgcacgcgccgcggttatgtcgagggtaaggacgccctcggccagccaacgaagacctggggtgaccttggcaagctgtgggctgagatcagcattccatctggccgcatgtacgaagccgcagcgcagatgcaggttcaggtcagcgctgagatcaacattcggtaccgcaaggacgtggtcgccggtcagcacctggtccacgacggcatcagctacgaaatcatcgccccgctggcaaccaaccagcgggacatgctcaaactcatgtgcaagacggtgaagcccaaatgagcaacggatcattgactgtcgtcggcctgggcgacctgcaggccgacttcgagcgcctggctcggtcggtgggcaacaaggtcgtgcgcgatgctgtcattgctggcgcgcgggttgcccgggacaagacgcggcaggcggccccattcaagaccggcaagctgaagaagaacattgaagccacccgcgtgaagcagggggaaacccctggcggagcgacggccggtgtccgcgtgaagaggccggccggcaaaacaagcaaacctcgcaagcgtccaggcaagacagggaagtcgaccacgaccgactacgacgcgccgttctactggcgatttctcgagtacggcacatcgaagatgcccgcagcgccgtttatccgccccacctgggatgccaacctggccgagatcgagaaggccaccgccgacaagctcgctgaaggcatcgacaacgcaatcacccggtaatccccatgattgagcaatccctcatcgccaggctctcgccgttggtggacgggcgcgttttctttggcgttgccccggccgatgccgagcagccgcgcctggtgatccagaccatcggcagcgatacagggttcaccctggccggctgggatggctccaaggacctcaccatccagctcgacgcctggggggagagcttccttcaggcgttgaccctggccggcgaggctttcgcggtcatgaccgccgacggcgatgacttcaccaccggcagcgcagatcgcctgccggacgttttcgaagatgacaccaagctcttcagcgtcagctgggagtacaccctgcaaccataggaggccccatggccgcgcagaacccaaccaaagcgaagttcgtcaaaacgcagggtacccagctcagcgtttccaagaccaccaccctcgacccggccgaggtcggcctcgagttcgcggacctctcggtcaccatcaagcaaccccagttccagggcggtcagtcggatgagatcgaagtgaccaccctggccagcgaggccaaggaatacaccgtgggcctggctgacaacggcaccttcagcatgtccggcaactggaaagctgacgatgaagcccagaccgtgctgcgcaccgcccgagatgatggcgagccgcgggcatttaagtcggtgttcaaggacggcacgtcctctgagttccttggcctggttacccagttcacctgggacgccgcacccaacggtaccgtcaatggcaccttcaacgtgcgcatcaccggcaaggtcaccttcaaagttcctccggtgactccgtaatggctcgccagaaagctgccgaaggcagcagcatccggcagaaggccctgcacccagtaagtaacttcaaacacgaagcagtaccagtgcctgagtggggcgagacggtgattgtgcgcgcaatgagcgccggcgactgggctgactaccgtcgccgttcactggagttgatcggcgccgcccgaaaggccgcaggcctgccagagatcggtgaggagagtgaatccgaggcagcgcagctcgatatcccggccgcgccaatctatgcacttgtactggttcgaaccctgttcgatgaatcgcttacccgtgtgttcaacgatgatgatgttggtgaggtagcggccgctttcagcccagtacacgatcgtctggttagtaaggcgtttgagctcagtggcgtgactgccgagcaggagccagaggtcgccgcgggaaacgactgaaaggagagccggatctagcttttatgctggctctggctctccgtctgggcaagaccctgcatgagctcaggtcggagatgtcggccgaagagctgctgctttggaaggcctataacgagcagtcgcccatcagtgatatgcgcggtgatgtgcaggctgcgatcaccgctgcagccgcgctgcaggcccagggcgcgaaagtctcggctgcggacatgcttccaacctggtcgagacctgcagaggagaccactgacgaggagcaggtcgaagagggcgaagagatgctgaaggcgtttctcttgggcaagaccgtgtcggcttgaagtttgggcggctagcagttgaggtgatacagtcgctccatttttcaggagggaaccctatgttgtggaaactaacgattttctcgcttgccgttgcggcaatagcaatttcgctatgcaagaaggtagcgaaagagcctggtaccgaaaatctactgagaactatcctctgcgcgtctttagtggtcgtgttgtttgcgtggtggtactttctctggtcaaaccctgagcgggcttcaggggcatacactgtcaattcggcagcactttctaaatactctgaagagcagtaccctcggttttataaaaactggggtgcggatggggtaaagagaattgaagtaaaggagcggcttgccttggataaaatatcgaggcaaaagaagtgcgattatgtttatgctgttggcttggcggaaagtcaaagtacgccacctaacaatataataatttatggcaattgcagtaatggctttcagttctacgtggggcccgatggaaatattctagcgttcaaaaaagttcactaacccgcttcggcgggttttttatgcccggagcaaacatgtcaggccaaacccttcgttcactgatcgtcagcgtcacagctgagactggtgcgtatcagcgtgaaatggcccgtgctggtcgtctcggtcagggttactttagaaccatcaccgatggtaaccggcaggctgtagccggatggaggtcacagcaggcggcaatcagcgcacaaaattctgctgtcagctcgctcacatccagcgtggggagttatgcagccgcaatggctggagcgctggctgtagggaacctgctaggtcgcgctgattcttggaattcaatctcggcacgaatcaaattggtaaccgccagcgccgacgattttaaaatggtgcaggaagggttgttcaatataagccaaaagactacctccctttatgctgataacgccaacttgtacacccgctcatcgcgagcccttaaagaatttggctactcaacccaagaagctgtcgattttactgaggccctagctaccagctttcaaatctccggttcaagtgctgacgaggtgacttcggttaccacacaattaagtcaagctctcgctaagggggctttacgagggcaagactttaacagtgtaagtcaaagtggcggccgcgcgatgcaggctctggctgatggcataggagtatccactggcgcgctaaaagcgatggcggacaatggcttattgactaccgacaagattgttactgctttgcttggtcagctaaagaagctccgagcagaatacgagcaaatgccgagcacaattagtggctcgatgaatactttggataacgccttcactaggtgggtcggtggtgtagatggtgctactgggagcacacaggcactttcaaaagtgatcgtttccctcggaagcaaccttgatactgttgccgcctctatccttgtggcaggtgcggcctacgcaggcctgaagctcggccagattgcccaggctatctggataaaagttcaggcccagcgaatcgagatcgctacccagatcggggcaaccaaggcccaagtcgacgccaccgccattgctgttcgcaaggcccaagcggacattctcggtgcgaggcatcaacttactttcgcaaccactactgcccaggctgcggctgcaaccagggcgctgtccgcggcgaggctcagtgaggtggttgccaccacggcgcacactcgcgctcttgctgcacatactgccgctgcatctttaagcgctcgggcgggcggggcgttgctgggcatgcttggcggtccagctggcctggtggccttggccgcgggcgctgccgctagcttcttcctgtttcgggacggcgcagaggaggcgaacactgcagcggtcgatctgaaaaagccgatcgcggacctgcgcaaggagtgggaagaactgggcaaagcccagcgccggccagtacttacaaaactgattgaggaacaggaagaggccaagcgcaaggccgctgaaattgttcgtgagatgcaggcggtttctcggggtccatccggtgattacctgggcggcaaacggtttggagccaatcagtttcagcgaaccgctgccgcggctaacttccgtcgcagcatcgttggtgggattgacatcgaccgcgccaccgaaacgctaagtggcgccatcaggcccaatcaagaggtcaaatcaaccctcgaggcccttgctgctcagtatcaggagagcatcggaaaggtcagcatcctgggtgatcagatcaacaccctgaatgacgtgatggccaaaggggaggacgctgcgaaagggttgggttccggcctggagagtattaaacccccggctcaggatgtagtcgacgcctggaagaagcgcatcgaaggtattaccgagcaaactgccaaactgaaagatgcttccaccttgggtgaagtgaatcggcagggggggcgagacggtctttcacaaacggctgaggggcgcgcgctgctggctcaggcgcaggccgctgctcgcctgagggacaccgaggagcaagccaagaaagctcgggaagagtcggcgcgcgtggcgaagcaagccgccgatgaggtcgagcgcaaagcgaaacaattgcaggacacttacagtcggacgctgaaatcactgcgagaacaggctgaggttcacgggcagaagactgaactcgccaaaatagagtttgagacgcgcaaggggtcgttgaaaaacattgatgcggccaagaaatcggagcttgagcgcgcagcaatcgctgtagaccacctcaacacccagaagtcgttcaaagagctgatgggggatgtgcagcgacaggaaaacagcttgctggcgactacccgtaagcgtaacgctgagcttgagcggatgcgcgcccaaggcggcctatcgtctgatcagtatcgaaagggcatcagtgcgatctccaaggcatcgattgaggatgcgcctcagttctccgggttggattcttcggtaaccggcgcctcgggcgagctggttaaaacggccgaggcggaagcccaactcaggaagtggcacagccgacagcttcagatgcagtctgaactacttgcggagaccttggccaaccaggaatccacgaacgagcaacggcttgcagctgaacagcgctacctggacagggtggcggacatcaacaggaccaacagccagcgcctcaccagcattcagaactcatacaaggtcgctgtcgtcggcacctttagcgagcttgcgggtcaggccgccgacatggtcgggaagattgccggcgagcaatctggggcttacaaggcgttgtttgttgcgcagaaggctttcgcggtcgcgtcgatcatcatgaacgcgcaaatcgcggcggccaaagcgccggctgagctgacagtgctgggtggcattccagtgggtgcggcgctgctggcggctggctacgcgaacgccggcatggtcgccggtatggccctggctggattttctagcggcggttataccggcgacggcggcaagttcgaacccaagggggtggttcacggtggggagttcgtcctgcgcaaggaagtggtgcagctgccgggcatgcgcgactacctcgaaggcctgaacaggcgcggctatgccactggcggctacgtcgggtcggctgctgcgcctgcttcgctcgggtattcaatgccacctgtcgccgatggcgctactgcagcgccgcgaatttccatccacatcagcggcgatggcacgggcggctcggttacatccactgagggctacgaggccatgggccaggccattctcaacacggtgcgccaagaaatgcccaaggttgcccggggcgtaatcatccaggagaagggccagaacggcctgcttgaccccagcaacaggaggaatgggtgatgcctgaagtattcacctggtccccgcgggtggggtcgagcggggacgtacaggccaatgtgctcacgtcccaatacaacaacggctacagccagcgcctgtcggtcgggatcaacaacctggctgggtctcaccaggtctcgttcacggggacggaggcctatctggcaccgattctggcgttcttcgttcgccacaagggcgcgatcagcttcttctggaagccacccttgcaagcccaggggcggtacatcaccacgggtggatggcagacggcgagccacggcaaggggcgatacacgctcagcaccacctttcaacaagtctttagtccatgaggtaaaacatgatcacggcagacgaccagaagcttgagcccggcgacctgatccagctgctcgagctggacggcgagtcgcggggtatgggcactttgcgttatcacgcgcatcaatgggatggcccgatttactggaaggggcaggcctacctgccaaggccgttcgaggtcggcggctttggccgtggcaccgagggcaacaccagcaccccaatgttgaaactgggcaacctcgacggcgtcatcacggccctgtgcgttcagttccaccacctggtggggatcaaggtcactgtccgcgagacgtacgccaagtacctcgatgcggccaacttccccggcggcaacccgacggcgggcgaccaggagcgcaccagtatttcgtttatcaacgtgccgaccagtatcggccggccggagattgtgttcggcctggcgccgccgacctcggtaaaggggcagatgctgccgggcggcttgatcatgaaccgctgcgagtggtgtctatggggtgagtaccgcg

SEQ ID NO: 5 - DNA, 1713 bp, unidentified
  source 1..1713: mol_type = unassigned DNA
gtggctaatttaaacagcgcgtcgtcatcaatcgatattctccaccatcggcgtgcaatggaacgttgggatatctttcgaagatataagcaaggcgaattacctatggacgtcgccatgcgagtcatgaatcttaagaagtctatgttttacaggctgttgggggttgtgaatagatctgctaactacgagtgcttactgcccggcaataaggggtgtaactctggttcgaggtacttaggaaataaggttgagaaactcatagatgatgcttatgaggatcattatgaaggatcgtctgcttcttttgctaatgtttggcgtcaactccaggcgataacaaaagtttctgacttgaaatgcccgagctaccatgcagtccgtatcagaattttagaaaaacctgaaatcgagaggttcaggaagaaatacggtgttgaagcagccgaccaaaagtactcgccccgtcctggcagtaagcaaaccaacaggccgttagagtgggtgcagattgatcacactttagcagacgtgatgttagtcgattcgcaggatcgaacccagcttatagggcgcccttgggtaacgctagcaatctgtaaacacacccggctgattctcggattttatctttctctcctgcatcccagtgctgtgagtgttgctatggtcattgggaattctgtggcgtcgaaatcatcgctgctaactaagttgggaattagtgaaaatgcactcccgcgccatggcttgatggagacaattcatacagacaatgcggctgaattcacctcagatatactcaggagcgcttgcgaatcacatgacataaaactagtgtctcggcgtcgcaagcattacggcggtcatatcgagagacttattggcaccatgatgaccactaaggttcactttctgagagggactacattctccaacgttctcaggcgccgtgactattctccagaaaaaaaagccgtactcacattccaggagttctgtaaggacttcgtagttaatgtgagtgtttataattctacaactcatagcgcgcttcaaaataaatcgccgaatcaagtgtgggacgaatattacactaaaaatccacgcccgaaaataatagactcatcggagctagaaagctttcgaatagatttcttcccgcaacgccttaaaaaaatacaaccctacggaattgaaattttggggcggcgctattatggcacgcccctgaaaggtttagtggggcgtgaagtcttggtgaagtttgacccatatgatcttacgcatgtatttgcgctgttgcaggggagctatcagctcataccgctatcttataattataagtcgcgcagtttggactatgagatgtatagatacgagagaaatcaaaaaggtgttaggaacggaacaattacggaggacgaggcgctaggcctcatgatcgaagctaaagcggacctggaagctgcgcaacaaaaaactcaggaagcgaaaaaggggaggaaatccgaggcgtctagaacccataaagctgcgaaggaaattataccggccaattcaattcctggttccattaatccgccactagctgtccagcatgatcggataggtattctcgactatctcatagcttcgcggcctgcagacacccatgcggaagatatcgactttagtagtcaaccaaaaatttatgatggagacttaaagtga

SEQ ID NO: 6 - DNA, 867 bp, unidentified
  source 1..867: mol_type = unassigned DNA
ttactggggaacacctgcctctttcgcaatttcatgaacggatcgcgctagagactgcttaatttgttgtaagtcgtcattattttttctcccaaatccaataacacaggctgccgcagcatcaacaaaaaaggtacttgcgatacgggtcatcattgtagaataggcccatgcttctttagccatattgaccttttgttcgatgggtatttcaagcgaaataagccacaaaatagtgtcttccccagtgagatggcttgcgccacttaaacgatggtagctttcgtagtaatcggtcttacgccccatcgcttcgaaacgcttaaatagcgactttggccactctgtgcttttatccacaggctcgattaaagcttgcgtctcaacatgacctacatatttttctagagattgaatgaagtcactcctctcatcaatcattgccaaaactttttccgcataactttcatctctgatcgtttccttccactcagaaagttttcgtccgtgctcatgcaaccaagacctaaaaaattgaatcaaagtgctagagtttccgattgtcgctaaatacatgatattcatggctccctctacaactacccttgcgagtgcttcagcgctggcaggggagcctgtagatatggcaaccaacataccttcagagtgctcgtgaatacgcccaagcaggtttatcaaactgtgaattctgaagctttctttagcattggaaagtttaacttcagacaggtactcggtgacaatattatttgtattataaattgcgtcaacagcaatcaatgagttttgaaggtcagcatggggggcgatatggaatttttttcgaaaatcttcaatatgactcac

SEQ ID NO: 7 - DNA, 1374 bp, unidentified
  source 1..1374: mol_type = unassigned DNA
atgcaatctctagcggcctatttacttgaacgaactgtaaactctgaagatgaaaaaatatcattaatagccgaaactagaaagcacttaagtaattggcttaaagaaaaaggagttgcagatcctgctggcagttcaggagaattcaaatccataagctcatctgaaaccggccactataagcgcgagaccgcagtaagcaacgatgaaatactggagcaaataagacttgaggagtcgcctagaaacaatcaaatattttttacaaatgtagcgttcgccacatccaaaacaagattttttgtatacattacactttcagccacgaccaaaaccagcattatctcccctatatcaattgatgctcgatgcccatcaattctgcgtgatatcttaagaaacggtactcagtggaaagtaggtaattacctagtgcctcacggtgatcgcgtacaaataaaaggcgatgaaaaaggcctcgaacttgcgcactatttaaagtcaagcacgcgaattttcccagttgtggttgtttccgaatacgaaggagagcaaatttggagagggcttggtcgaaagatcgcccatgaccttgctggcctagctcaaatttacgaagtggatgacaaagcctcttgggctattacagatgtaattgaaaagcaaaactcttgttatagcggcgctataaggctttattggccgagcaatggatccagctcagttgagcagttccatggaaccttgtggacgccatacaaattattatctaatgataaggacggggaagcagaagctagatttcgtagacaaatccgccgacgtgtcatgagcgtatctgcacttactattttgccaccaaaagaaattcatgaaattcagagcgctagtgctcgtaagcggttaaccgatttagaaggtaaagcatcatccaccgacgacttagtggaattggctcaatcatatctcgatgatgccgatacgctccgatctgagaacacagagcttcaagaaaaactatctttagcgataactcgcgcagagaatgcggaagcaatcgctgaaaacatttcaagaccactgcaagagtttgacaccgaagcccccacagaaaatggtgatgatgagcaagaggaacaagacctctctccacccgtgccaggagagataagatactacaagaaagtccgtaacactccttctcatgaccttctaacgcacgtcgctgattgtaagcatacgagttggcaagctgcccacaaagctgaaaaagcgaagaaaggagtggagaaacttgaaggtgtcagcaattgggatgtaatacatcattgcggaacgtgtaaggggggaggaatgtggagagttaaatggtga

SEQ ID NO: 8 - DNA, 1140 bp, unidentified
  source 1..1140: mol_type = unassigned DNA
atgattcttaagtcagttgaatattatgagggtagtaagacaccgcagttttgggcgttagataggcttgacctaggtaagaggaatttggttgtaggcaaaaactctactggtaagacgcgcgctttaaacgtgatagttggattggcgagaattatttctactgctggaagtttgcctgattcggcaagatatgatgccacttgggaggataagagtggtaaggtttttcgatatcaactctctctcgagtcgagctcggtacagtcggaagttctttcaatcgatggacaggttgttttggatcgctcggctgggggggtaggtcgaatatgggctgagcaagtttctaacggttcaataattccttttcaaacacctaccaatgagctgtctgtactaaagcgccgggattctttgcagcacggctttatagagccattatataaatgggcttcgcaggttcgtcattacaacttcggttctagtttagggaaagatcatcttacatttatttctccatctgcacctgccgtagatgaaaaagatcagaatcaggttgtaggtatttttagaaaggggaagaaagagtttggcgctgattttataaatgctatcaagtccgatatggcgcgtattggttatccgttagatgatgtgacgacaggagcaccttacactgtgagagttgaaaacgctccaggtgaggttgcttccatactagttcgcgaaacaggtcttatgggagtaactgatagcttcggcatgtcccaagggatgtatcgagtgttagctttagttattcatatgaattacctgcaatttaatcgtgttagtacctgtgtagtcgtcgacgatgtgggtgagggtctggattatgaaagatcctgcgatatcattcatctgctgcgagaaaaatcggaagcctcagacctgcaaattataatgtcaaccaacgatcgtttcgttatgaacgaggttcccctgcaagagtggactgtgcttcatcgatatggtgcgaaggttgaggttagtaactatgggaattccaaagatctgtttgatgacttcaagttcacagggttaagcaatttttccttctttgaaatggattttttaaaagaatctcgcggagattga

SEQ ID NO: 9 - DNA, 408 bp, unidentified
  source 1..408: mol_type = unassigned DNA
atgtcacacccagaaaatagcacccagctatctaatccgcaagacacccactcggatatcagggggatcatctacctcatggtctgtgcagataccgaggatatctcgtaccaatgggagccgttcctgcagaaaggactggccatcgaacttcttgagatgctggcgccagagtttccgggagcacggatgcgtttgatccagtgcgccggacttgtttcggatcttgaatccgttttgggggcggctgagcgccagaaggacttgatcattagttgccggaacgccatgcgacctggccgcacataccttgagcgaatggccgcgaagcgaatcccaatgcccgcgccacaaaacctaacctctcaagttcgtggcgcggaggttacccaatgccaaggccaatga

SEQ ID NO: 10 - DNA, 708 bp, unidentified
  source 1..708: mol_type = unassigned DNA
atgcgacggattgctttttttgtagagggctactcggaattattatttgtagataagcttcttgtggaaattgccggggcacataatgtcgctatcgagcaaaggcagattagtggtggagttagggttccacgttctgtcaaggtaatccaggcggctaatattgatgctggccaacaatattatgtgcttatcgtggattgtggaggggagtcgcaagtgaagacacgacttcaggaggagcatgaggggcttactaggcaagggtacgaaaaaataatctgtatccgggatgttcgtcctgagtttactcgagaggaaattcctaggctagagcgagggatgcgcttgtatgtaaaagggagtcttgctccggtagactttatcttgactacgatggagctagaagcttggtttttggcggagttcaatcactacccaaaaattgacccggcattaaactctgaagctgttcacgagcttcttggataccatcctgaaacagatgatcctgggactcgagactgccccgctgacgatttgcggtcatgctacgctattgctggaaagacatacgaaaaatcagaagcaatccggacggtggaagctctggactatttatatgtttataccgacctgaaggatagaattcccgaagtgggccgaatagttgcccacgtcgatgagtttttaacaccttcatcctga

SEQ ID NO: 11 - DNA, 2778 bp, unidentified
  source 1..2778: mol_type = unassigned DNA
atgcaggctctggctgatggcataggagtatccactggcgcgctaaaagcgatggcggacaatggcttattgactaccgacaagattgttactgctttgcttggtcagctaaagaagctccgagcagaatacgagcaaatgccgagcacaattagtggctcgatgaatactttggataacgccttcactaggtgggtcggtggtgtagatggtgctactgggagcacacaggcactttcaaaagtgatcgtttccctcggaagcaaccttgatactgttgccgcctctatccttgtggcaggtgcggcctacgcaggcctgaagctcggccagattgcccaggctatctggataaaagttcaggcccagcgaatcgagatcgctacccagatcggggcaaccaaggcccaagtcgacgccaccgccattgctgttcgcaaggcccaagcggacattctcggtgcgaggcatcaacttactttcgcaaccactactgcccaggctgcggctgcaaccagggcgctgtccgcggcgaggctcagtgaggtggttgccaccacggcgcacactcgcgctcttgctgcacatactgccgctgcatctttaagcgctcgggcgggcggggcgttgctgggcatgcttggcggtccagctggcctggtggccttggccgcgggcgctgccgctagcttcttcctgtttcgggacggcgcagaggaggcgaacactgcagcggtcgatctgaaaaagccgatcgcggacctgcgcaaggagtgggaagaactgggcaaagcccagcgccggccagtacttacaaaactgattgaggaacaggaagaggccaagcgcaaggccgctgaaattgttcgtgagatgcaggcggtttctcggggtccatccggtgattacctgggcggcaaacggtttggagccaatcagtttcagcgaaccgctgccgcggctaacttccgtcgcagcatcgttggtgggattgacatcgaccgcgccaccgaaacgctaagtggcgccatcaggcccaatcaagaggtcaaatcaaccctcgaggcccttgctgctcagtatcaggagagcatcggaaaggtcagcatcctgggtgatcagatcaacaccctgaatgacgtgatggccaaaggggaggacgctgcgaaagggttgggttccggcctggagagtattaaacccccggctcaggatgtagtcgacgcctggaagaagcgcatcgaaggtattaccgagcaaactgccaaactgaaagatgcttccaccttgggtgaagtgaatcggcagggggggcgagacggtctttcacaaacggctgaggggcgcgcgctgctggctcaggcgcaggccgctgctcgcctgagggacaccgaggagcaagccaagaaagctcgggaagagtcggcgcgcgtggcgaagcaagccgccgatgaggtcgagcgcaaagcgaaacaattgcaggacacttacagtcggacgctgaaatcactgcgagaacaggctgaggttcacgggcagaagactgaactcgccaaaatagagtttgagacgcgcaaggggtcgttgaaaaacattgatgcggccaagaaatcggagcttgagcgcgcagcaatcgctgtagaccacctcaacacccagaagtcgttcaaagagctgatgggggatgtgcagcgacaggaaaacagcttgctggcgactacccgtaagcgtaacgctgagcttgagcggatgcgcgcccaaggcggcctatcgtctgatcagtatcgaaagggcatcagtgcgatctccaaggcatcgattgaggatgcgcctcagttctccgggttggattcttcggtaaccggcgcctcgggcgagctggttaaaacggccgaggcggaagcccaactcaggaagtggcacagccgacagcttcagatgcagtctgaactacttgcggagaccttggccaaccaggaatccacgaacgagcaacggcttgcagctgaacagcgctacctggacagggtggcggacatcaacaggaccaacagccagcgcctcaccagcattcagaactcatacaaggtcgctgtcgtcggcacctttagcgagcttgcgggtcaggccgccgacatggtcgggaagattgccggcgagcaatctggggcttacaaggcgttgtttgttgcgcagaaggctttcgcggtcgcgtcgatcatcatgaacgcgcaaatcgcggcggccaaagcgccggctgagctgacagtgctgggtggcattccagtgggtgcggcgctgctggcggctggctacgcgaacgccggcatggtcgccggtatggccctggctggattttctagcggcggttataccggcgacggcggcaagttcgaacccaagggggtggttcacggtggggagttcgtcctgcgcaaggaagtggtgcagctgccgggcatgcgcgactacctcgaaggcctgaacaggcgcggctatgccactggcggctacgtcgggtcggctgctgcgcctgcttcgctcgggtattcaatgccacctgtcgccgatggcgctactgcagcgccgcgaatttccatccacatcagcggcgatggcacgggcggctcggttacatccactgagggctacgaggccatgggccaggccattctcaacacggtgcgccaagaaatgcccaaggttgcccggggcgtaatcatccaggagaagggccagaacggcctgcttgaccccagcaacaggaggaatgggtga

SEQ ID NO: 12 - DNA, 447 bp, unidentified
  source 1..447: mol_type = unassigned DNA
atggctcgccagaaagctgccgaaggcagcagcatccggcagaaggccctgcacccagtaagtaacttcaaacacgaagcagtaccagtgcctgagtggggcgagacggtgattgtgcgcgcaatgagcgccggcgactgggctgactaccgtcgccgttcactggagttgatcggcgccgcccgaaaggccgcaggcctgccagagatcggtgaggagagtgaatccgaggcagcgcagctcgatatcccggccgcgccaatctatgcacttgtactggttcgaaccctgttcgatgaatcgcttacccgtgtgttcaacgatgatgatgttggtgaggtagcggccgctttcagcccagtacacgatcgtctggttagtaaggcgtttgagctcagtggcgtgactgccgagcaggagccagaggtcgccgcgggaaacgactga

SEQ ID NO: 13 - DNA, 303 bp, unidentified
  source 1..303: mol_type = unassigned DNA
atgctggctctggctctccgtctgggcaagaccctgcatgagctcaggtcggagatgtcggccgaagagctgctgctttggaaggcctataacgagcagtcgcccatcagtgatatgcgcggtgatgtgcaggctgcgatcaccgctgcagccgcgctgcaggcccagggcgcgaaagtctcggctgcggacatgcttccaacctggtcgagacctgcagaggagaccactgacgaggagcaggtcgaagagggcgaagagatgctgaaggcgtttctcttgggcaagaccgtgtcggcttga

SEQ ID NO: 14 - DNA, 1077 bp, unidentified
  source 1..1077: mol_type = unassigned DNA
atggatcagcctgaagttgagaaaaggcaggagcagccgcccatcaccgtaccgccgagttgtcagataatttttcaatccttgcctgataatgtcgagtggaactctaagtttcaggaaataattcgccagtatgttcttgaagttagccgatacatcgatctcgctattattgataatataactattgggttcgattacgattttgcgataagttcggttgagcttggttatgaatcggcgcgagcaaagcagtacactaattcaaacggattggtcggcgttggtaaaaccctgaaggtcgttcgtgatggtgagctcaaggttcatgttgtcttaaacgcaaactatctgactaggctagtggacttcgaaacagacgttaacggcttttggcaggatggtaatctccttgcgcacgaactagcccacgtcgaagtgataagctggtttcagcagcattctccaggtgttcttctttccaagtgggagggtgactgggctttagcgtgtatgcgtgatgcggcccatactatctgggaggagtacgcggcttgcgctctgagcgctatctttagcaaaggtgacgcagtcacagataccatgattagcgggctggaaacttctatttctggggcggtagagcgtgctagggatgcgattaaagtgtaccggacacaatcaaatgtagatgatcttctgtcagcggtgggtgctgaagttgctacccctctgaaaatggccgcttacctgcttggtcatttggatggctcggggcaggagctaaatctagttgagcggtcaccaaatacagaaagtagtttgtttggccggcatattccaaatttgcagaattccttgcgtaaggcgtgggaaactcgtgagtcctggaaaggtatggaaggggttgatggtatcgtggaggttattgtaagcacaatgcaggatgtaggcctaatactcactctaaatcctgctgggtctaaagttgatgtgccatttactgccgagacgatgccaaacggcgaggcggacatgcaggcgattcgcattgctcaggttcttggcttgcgatga

SEQ ID NO: 15 - DNA, 714 bp, unidentified
  source 1..714: mol_type = unassigned DNA
atgcccacagaaaaccgatccagcaacaccgaacaggtggtcagcatcccccgcgactgggccgagaactacgcaggccttctggaggaccgctgcgcctacgtgcgggccgaacaggtaaacgcacttctggcccagccagccgcccagcaccagggcgagcaattcacctacagctcaaagcaagcaaccaattgcgctggctgcggcactcgcaagcacacgccgttgcgagtggatgaaatgggcggctatgtgtgcttgacctgtatcgaccaaaaacttgaatctctgctgccgtcgcaagagcaccagggcaagccggtggcatatctcgtcactgatgttcacggtcaaaagaaggctctccgcgccggagccgaaggcattgaaaggcatcgccattcaggctctaccctggtaccgctctacagccacgccgatgctggcgaggttgagcgctggaaggagcttcatgccgccatgcagttgcagcggaaccaccaccgtgaacgagccgacaccctgcgcgcccagctgaccgaactgcgggacatgctggacgaactctactttgctcaggacgggcatattccgcgcatcgaagccgccctatccgccagcgcagagccgagctcgccggttgagcgcgaccagggcatacctggcacctccttccagcgcctgaacatgctcgccaatcagggcgaatga

SEQ ID NO: 16 - DNA, 882 bp, unidentified
  source 1..882: mol_type = unassigned DNA
tcaccgttgcgctgcttcggtttcaacgaaagcgtcggcttgcagatcgataatttgctgcggcccgtactggtagctgagcttcagtaattcgctccagtcccaagcgatagaggagttcagctcgttacggatcttcaaatcatggaaagcattttgctcccaacccatgtaacgcttaccggcatacagctttgaacccgtagctaccaactgctgaacagcggcatcccactcctcctgaagccgctcggtggccaggcggaccgctgaccgttctatcttttccgattcgcggactgcctcttcaatatgttcgtcaattagcttgatctcttgctccaatgccgagacgatcaggccttgacggcgttgctgctcgagctcggttgccaggactttggcagctttctgcacatcagcagcggctgtctcttcgccatcagcatcgccccaagcgacagcttgtgcatacgcgcgagcagcctcctcctcagcttgacgggcattggtgatcgcctgctcgttatgagctcggacctcctccagtcgcgtgctcagcgttttccttttgccatgaaggtcggccttgtccaacgaccagttctccatcttttccttgtagtcggccatcaactcgacgctattggctttgcgctcgatccaggcaatgctttgatcaacgacggagattttgtgttcgatatcccctacttttgattccgcatttcgcacgctgatccgcagatcttcaccggctggagtttcagcaaagccagggatactcagctgctcttcccatcgagcaatttgcccttcgagctcactaatctctgcttcgtgtttgctgcgttcggtgttcagtttttcgaggttttgcat

SEQ ID NO: 17 - DNA, 780 bp, unidentified
  source 1..780: mol_type = unassigned DNA
gtgagcgccaagccaaaagcgccgcagagcgctgcgcaactgctcaaagtggcgggcgccaccagcgacttgcggggcgcagtcataagtcatcaggcgccaccacctccggctagccccaaagctctgcctccgggctcggttgatgttgtgaacacgttattcaaagagctgcaggccattttccctgcctggaagcaggcctggccggataccgaatcacttcggactgcaaagcgcagctggatcaaggccttcattgcggagggtatcaaccagctggaacaaatccgatatggcgttgagcgctgcagatcccttggcaccgacttcgcgcccagcgtcggtaagttcatcaagctgtgccagccaacccccgagatgctcggcattccacctcacgacaaggcgttccgcgaggcgctggtgaatgctcaccctagccggttcggcagtcgcgtttggtctcaccctgcgatccgccacgcagccctgcagtgcgagctgcacaatctgggcgacctagcccccgacaaggcttgcgcgattttcgatcgtgcctatgacgtcaccatccgcctgctggtgcagggtaaggcgctggaagatatcgcaatcggcatcgggtacgacgggcagaaaaccgaggcggagctggctgacgagcatggccagtggcgtcagcagcaaatcatggcccgtcaggccatcccggcaaatggccaggatgcccgccgcgcgctgctggcccgctttggattggggctcgagcatgactga